European Patent Application EP 4 725 501 A1, published April 15, 2026. Title: 特异性结合MASP3的抗体以及特异性结合MASP3和MASP2的多特异性抗体. Applicant: 舒泰神（北京）生物制药股份有限公司. Application CN. The sequence listing filed with the application follows.

SEQUENCE LISTING (76 sequences)

SEQ ID NO: 1 - protein, 5 aa, synthetic construct
GKWIE

SEQ ID NO: 2 - protein, 17 aa, synthetic construct
EILPGSGSTDYNERFKD

SEQ ID NO: 3 - protein, 4 aa, synthetic construct
SEDL

SEQ ID NO: 4 - protein, 17 aa, synthetic construct
KSSQSLLNSVTRKTYLA

SEQ ID NO: 5 - protein, 17 aa, synthetic construct
KSSQNLFNSRTRKNYLA

SEQ ID NO: 6 - protein, 7 aa, synthetic construct
WASTRES

SEQ ID NO: 7 - protein, 8 aa, synthetic construct
KQSYTLPT

SEQ ID NO: 8 - protein, 8 aa, synthetic construct
KQSYIPFT

SEQ ID NO: 9 - protein, 17 aa, synthetic construct
  VARIANT 5: note = X is N or S
  VARIANT 7: note = X is F or L
  VARIANT 10: note = X is R or V
  VARIANT 14: note = X is N or T
KSSQXLXNSXTRKXYLA

SEQ ID NO: 10 - protein, 8 aa, synthetic construct
  VARIANT 5: note = X is I or T
  VARIANT 6: note = X is L or P
  VARIANT 7: note = X is F or P
KQSYXXXT

SEQ ID NO: 11 - protein, 113 aa, synthetic construct
EVQLQQSGAELVKPGASVKISCKASGYTFTGKWIEWVKQRPGHGLEWIGEILPGSGSTDYNERFKDKATFTADTSSNTAYMQLTSLTPDDSATYYCVRSEDLWGSGTTLTVSS

SEQ ID NO: 12 - protein, 113 aa, synthetic construct
QVQLVQSGAEVKKPGASVKVSCKASGYTFTGKWIEWVRQAPGQGLEWIGEILPGSGSTDYNERFKDRATFTADTSTSTAYMELSSLRSEDTAVYYCVRSEDLWGQGTLVTVSS

SEQ ID NO: 13 - protein, 113 aa, synthetic construct
QVQLVQSGAEVKKPGASVKVSCKASGYTFTGKWIEWVRQAPGQGLEWMGEILPGSGSTDYNERFKDRATFTADTSTSTAYMELSSLRSEDTAVYYCVRSEDLWGQGTLVTVSS

SEQ ID NO: 14 - protein, 113 aa, synthetic construct
QVQLVQSGAEVKKPGASVKVSCKASGYTFTGKWIEWVRQAPGQGLEWMGEILPGSGSTDYNERFKDRVTFTADTSTSTVYMELSSLRSEDTAVYYCVRSEDLWGQGTLVTVSS

SEQ ID NO: 15 - protein, 113 aa, synthetic construct
QVQLVQSGAEVKKPGASVKVSCKASGYTFTGKWIEWVRQAPGQGLEWIGEILPGSGSTDYNERFKDRATFTADTSTSTVYMELSSLRSEDTAVYYCVRSEDLWGQGTLVTVSS

SEQ ID NO: 16 - protein, 112 aa, synthetic construct
DVVMTQTPSSLAVSAGEKVTMSCKSSQSLLNSVTRKTYLAWYQQKPGQSPKLLIYWASTRESGVPDRFTGSGSGTDFTLTISSVQAEDLAIYYCKQSYTLPTFGGGTKLEIK

SEQ ID NO: 17 - protein, 112 aa, synthetic construct
DIVMTQSPDSLAVSLGERATINCKSSQSLLNSVTRKTYLAWYQQKPGQPPKLLIYWASTRESGVPDRFSGSGSGTDFTLTISSLQAEDVAVYYCKQSYTLPTFGGGTKVEIK

SEQ ID NO: 18 - protein, 112 aa, synthetic construct
DIVMTQSPDSLAVSLGERATINCKSSQSLLNSVTRKTYLAWYQQKPGQSPKLLIYWASTRESGVPDRFSGSGSGTDFTLTISSLQAEDVAVYYCKQSYTLPTFGGGTKVEIK

SEQ ID NO: 19 - protein, 112 aa, synthetic construct
DIVLTQSPSSLAVSAGEKVTMTCKSSQNLFNSRTRKNYLAWFQQKPGQSPKLLIYWASTRESGVPDRFTGSGSGTDFTLTISSVQAEDLAVYYCKQSYIPFTFGGGTKLEIK

SEQ ID NO: 20 - protein, 112 aa, synthetic construct
EIVLTQSPATLSVSPGERATLSCKSSQNLFNSRTRKNYLAWFQQKPGQSPRLLIYWASTRESGIPARFSGSGSGTEFTLTISSLQSEDFAVYYCKQSYIPFTFGGGTKVEIK

SEQ ID NO: 21 - protein, 112 aa, synthetic construct
DIVLTQSPDSLAVSLGERATINCKSSQNLFNSRTRKNYLAWFQQKPGQSPKLLIYWASTRESGVPDRFSGSGSGTDFTLTISSLQAEDVAVYYCKQSYIPFTFGGGTKVEIK

SEQ ID NO: 22 - protein, 112 aa, synthetic construct
DIVMTQSPDSLAVSLGERATINCKSSQNLFNSRTRKNYLAWFQQKPGQSPKLLIYWASTRESGVPDRFSGSGSGTDFTLTISSLQAEDVAVYYCKQSYIPFTFGGGTKVEIK

SEQ ID NO: 23 - protein, 6 aa, synthetic construct
SDYAWN

SEQ ID NO: 24 - protein, 16 aa, synthetic construct
YISYSGRTSYNPSLKS

SEQ ID NO: 25 - protein, 5 aa, synthetic construct
HYGDY

SEQ ID NO: 26 - protein, 11 aa, synthetic construct
KASQNVGTNVA

SEQ ID NO: 27 - protein, 7 aa, synthetic construct
SASYRYS

SEQ ID NO: 28 - protein, 9 aa, synthetic construct
HQYNSNPLT

SEQ ID NO: 29 - protein, 9 aa, synthetic construct
HQYNANPLT

SEQ ID NO: 30 - protein, 9 aa, synthetic construct
HQYNENPLT

SEQ ID NO: 31 - protein, 9 aa, synthetic construct
HQYQSNPLT

SEQ ID NO: 32 - protein, 9 aa, synthetic construct
HQYSSNPLT

SEQ ID NO: 33 - protein, 9 aa, synthetic construct
  VARIANT 4: note = X is N, Q or S
  VARIANT 5: note = X is A, E or S
HQYXXNPLT

SEQ ID NO: 34 - protein, 114 aa, synthetic construct
QVQLQESGPGLVKPSETLSLTCTVSGYSITSDYAWNWIRQPPGKKLEWMGYISYSGRTSYNPSLKSRITISRDTSKNQFSLKLSSVTAADTAVYYCSRHYGDYWGQGTLVTVSS

SEQ ID NO: 35 - protein, 114 aa, synthetic construct
EVKLQESGPGLVKPSQSLSLTCTVTGYSITSDYAWNWIRQFPGNKLEWMGYISYSGRTSYNPSLKSRISITRDTSNNQFFLQLNSVTTEDTATYYCSRHYGDYWGQGTTLTVSS

SEQ ID NO: 36 - protein, 107 aa, synthetic construct
EIVMTQSPATLSVSPGERATLSCKASQNVGTNVAWYQQKPGQSPRALIYSASYRYSGIPARFSGSGSGTEFTLTISSLQSEDFAVYFCHQYNSNPLTFGGGTKVEIK

SEQ ID NO: 37 - protein, 107 aa, synthetic construct
EIVMTQSPATLSVSPGERATLSCKASQNVGTNVAWYQQKPGQSPRALIYSASYRYSGIPARFSGSGSGTEFTLTISSLQSEDFAVYFCHQYNANPLTFGGGTKVEIK

SEQ ID NO: 38 - protein, 107 aa, synthetic construct
EIVMTQSPATLSVSPGERATLSCKASQNVGTNVAWYQQKPGQSPRALIYSASYRYSGIPARFSGSGSGTEFTLTISSLQSEDFAVYFCHQYNENPLTFGGGTKVEIK

SEQ ID NO: 39 - protein, 107 aa, synthetic construct
EIVMTQSPATLSVSPGERATLSCKASQNVGTNVAWYQQKPGQSPRALIYSASYRYSGIPARFSGSGSGTEFTLTISSLQSEDFAVYFCHQYQSNPLTFGGGTKVEIK

SEQ ID NO: 40 - protein, 107 aa, synthetic construct
EIVMTQSPATLSVSPGERATLSCKASQNVGTNVAWYQQKPGQSPRALIYSASYRYSGIPARFSGSGSGTEFTLTISSLQSEDFAVYFCHQYSSNPLTFGGGTKVEIK

SEQ ID NO: 41 - protein, 107 aa, synthetic construct
DIVMTQSPATLSVSPGERATLSCKASQNVGTNVAWYQQKPGQSPRALIYSASYRYSGIPARFSGSGSGTEFTLTISSLQSEDFAVYFCHQYNANPLTFGGGTKVEIK

SEQ ID NO: 42 - protein, 107 aa, synthetic construct
DILMTQTPKFMSTSVGDRVSVTCKASQNVGTNVAWYQQKPGQSPKALIYSASYRYSGVPDRFTGSGSGTDFTLTISNVQSEDLAEYFCHQYNSNPLTFGAGTKLELK

SEQ ID NO: 43 - protein, 330 aa, synthetic construct
ASTKGPSVFPLAPSSKSTSGGTAALGCLVKDYFPEPVTVSWNSGALTSGVHTFPAVLQSSGLYSLSSVVTVPSSSLGTQTYICNVNHKPSNTKVDKKVEPKSCDKTHTCPPCPAPELLGGPSVFLFPPKPKDTLMISRTPEVTCVVVDVSHEDPEVKFNWYVDGVEVHNAKTKPREEQYNSTYRVVSVLTVLHQDWLNGKEYKCKVSNKALPAPIEKTISKAKGQPREPQVYTLPPSREEMTKNQVSLTCLVKGFYPSDIAVEWESNGQPENNYKTTPPVLDSDGSFFLYSKLTVDKSRWQQGNVFSCSVMHEALHNHYTQKSLSLSPGK

SEQ ID NO: 44 - protein, 327 aa, synthetic construct
ASTKGPSVFPLAPCSRSTSESTAALGCLVKDYFPEPVTVSWNSGALTSGVHTFPAVLQSSGLYSLSSVVTVPSSSLGTKTYTCNVDHKPSNTKVDKRVESKYGPPCPSCPAPEFLGGPSVFLFPPKPKDTLMISRTPEVTCVVVDVSQEDPEVQFNWYVDGVEVHNAKTKPREEQFNSTYRVVSVLTVLHQDWLNGKEYKCKVSNKGLPSSIEKTISKAKGQPREPQVYTLPPSQEEMTKNQVSLTCLVKGFYPSDIAVEWESNGQPENNYKTTPPVLDSDGSFFLYSRLTVDKSRWQEGNVFSCSVMHEALHNHYTQKSLSLSLGK

SEQ ID NO: 45 - protein, 107 aa, synthetic construct [sequence omitted]

SEQ ID NO: 46 - protein, 106 aa, synthetic construct
GQPKAAPSVTLFPPSSEELQANKATLVCLISDFYPGAVTVAWKADSSPVKAGVETTTPSKQSNNKYAASSYLSLTPEQWKSHRSYSCQVTHEGSTVEKTVAPTECS

SEQ ID NO: 47 - protein, 217 aa, synthetic construct
APELLGGPSVFLFPPKPKDTLMISRTPEVTCVVVDVSHEDPEVKFNWYVDGVEVHNAKTKPREEQYNSTYRVVSVLTVLHQDWLNGKEYKCKVSNKALPAPIEKTISKAKGQPREPQVYTLPPSREEMTKNQVSLTCLVKGFYPSDIAVEWESNGQPENNYKTTPPVLDSDGSFFLYSKLTVDKSRWQQGNVFSCSVMHEALHNHYTQKSLSLSPGK

SEQ ID NO: 48 - protein, 217 aa, synthetic construct
APEFLGGPSVFLFPPKPKDTLMISRTPEVTCVVVDVSQEDPEVQFNWYVDGVEVHNAKTKPREEQFNSTYRVVSVLTVLHQDWLNGKEYKCKVSNKGLPSSIEKTISKAKGQPREPQVYTLPPSQEEMTKNQVSLTCLVKGFYPSDIAVEWESNGQPENNYKTTPPVLDSDGSFFLYSRLTVDKSRWQEGNVFSCSVMHEALHNHYTQKSLSLSLGK

SEQ ID NO: 49 - protein, 98 aa, synthetic construct
ASTKGPSVFPLAPSSKSTSGGTAALGCLVKDYFPEPVTVSWNSGALTSGVHTFPAVLQSSGLYSLSSVVTVPSSSLGTQTYICNVNHKPSNTKVDKKV

SEQ ID NO: 50 - protein, 98 aa, synthetic construct
ASTKGPSVFPLAPCSRSTSESTAALGCLVKDYFPEPVTVSWNSGALTSGVHTFPAVLQSSGLYSLSSVVTVPSSSLGTKTYTCNVDHKPSNTKVDKRV

SEQ ID NO: 51 - protein, 221 aa, synthetic construct
QVQLQESGPGLVKPSETLSLTCTVSGYSITSDYAWNWIRQPPGKKLEWMGYISYSGRTSYNPSLKSRITISRDTSKNQFSLKLSSVTAADTAVYYCSRHYGDYWGQGTLVTVSSASVAAPSVFIFPPSDEQLKSGTASVVCLLNNFYPREAKVQWKVDNALQSGNSQESVTEQDSKDSTYSLSSTLTLSKADYEKHKVYACEVTHQGLSSPVTKSFNRGEC

SEQ ID NO: 52 - protein, 212 aa, synthetic construct
EIVMTQSPATLSVSPGERATLSCKASQNVGTNVAWYQQKPGQSPRALIYSASYRYSGIPARFSGSGSGTEFTLTISSLQSEDFAVYFCHQYNANPLTFGGGTKVEIKSSASTKGPSVFPLAPSSKSTSGGTAALGCLVKDYFPEPVTVSWNSGALTSGVHTFPAVLQSSGLYSLSSVVTVPSSSLGTQTYICNVNHKPSNTKVDKKVEPKSC

SEQ ID NO: 53 - protein, 211 aa, synthetic construct
QVQLVQSGAEVKKPGASVKVSCKASGYTFTGKWIEWVRQAPGQGLEWMGEILPGSGSTDYNERFKDRVTFTADTSTSTVYMELSSLRSEDTAVYYCVRSEDLWGQGTLVTVSSASTKGPSVFPLAPSSKSTSGGTAALGCLVKDYFPEPVTVSWNSGALTSGVHTFPAVLQSSGLYSLSSVVTVPSSSLGTQTYICNVNHKPSNTKVDKKV

SEQ ID NO: 54 - protein, 219 aa, synthetic construct
EIVLTQSPATLSVSPGERATLSCKSSQNLFNSRTRKNYLAWFQQKPGQSPRLLIYWASTRESGIPARFSGSGSGTEFTLTISSLQSEDFAVYYCKQSYIPFTFGGGTKVEIKRTVAAPSVFIFPPSDEQLKSGTASVVCLLNNFYPREAKVQWKVDNALQSGNSQESVTEQDSKDSTYSLSSTLTLSKADYEKHKVYACEVTHQGLSSPVTKSFNRGEC

SEQ ID NO: 55 - protein, 211 aa, synthetic construct
QVQLVQSGAEVKKPGASVKVSCKASGYTFTGKWIEWVRQAPGQGLEWIGEILPGSGSTDYNERFKDRATFTADTSTSTAYMELSSLRSEDTAVYYCVRSEDLWGQGTLVTVSSASTKGPSVFPLAPSSKSTSGGTAALGCLVKDYFPEPVTVSWNSGALTSGVHTFPAVLQSSGLYSLSSVVTVPSSSLGTQTYICNVNHKPSNTKVDKKV

SEQ ID NO: 56 - protein, 219 aa, synthetic construct
DIVLTQSPDSLAVSLGERATINCKSSQNLFNSRTRKNYLAWFQQKPGQSPKLLIYWASTRESGVPDRFSGSGSGTDFTLTISSLQAEDVAVYYCKQSYIPFTFGGGTKVEIKRTVAAPSVFIFPPSDEQLKSGTASVVCLLNNFYPREAKVQWKVDNALQSGNSQESVTEQDSKDSTYSLSSTLTLSKADYEKHKVYACEVTHQGLSSPVTKSFNRGEC

SEQ ID NO: 57 - protein, 211 aa, synthetic construct
QVQLVQSGAEVKKPGASVKVSCKASGYTFTGKWIEWVRQAPGQGLEWMGEILPGSGSTDYNERFKDRATFTADTSTSTAYMELSSLRSEDTAVYYCVRSEDLWGQGTLVTVSSASTKGPSVFPLAPSSKSTSGGTAALGCLVKDYFPEPVTVSWNSGALTSGVHTFPAVLQSSGLYSLSSVVTVPSSSLGTQTYICNVNHKPSNTKVDKKV

SEQ ID NO: 58 - protein, 219 aa, synthetic construct
DIVMTQSPDSLAVSLGERATINCKSSQNLFNSRTRKNYLAWFQQKPGQSPKLLIYWASTRESGVPDRFSGSGSGTDFTLTISSLQAEDVAVYYCKQSYIPFTFGGGTKVEIKRTVAAPSVFIFPPSDEQLKSGTASVVCLLNNFYPREAKVQWKVDNALQSGNSQESVTEQDSKDSTYSLSSTLTLSKADYEKHKVYACEVTHQGLSSPVTKSFNRGEC

SEQ ID NO: 59 - protein, 448 aa, synthetic construct
QVQLQESGPGLVKPSETLSLTCTVSGYSITSDYAWNWIRQPPGKKLEWMGYISYSGRTSYNPSLKSRITISRDTSKNQFSLKLSSVTAADTAVYYCSRHYGDYWGQGTLVTVSSASVAAPSVFIFPPSDEQLKSGTASVVCLLNNFYPREAKVQWKVDNALQSGNSQESVTEQDSKDSTYSLSSTLTLSKADYEKHKVYACEVTHQGLSSPVTKSFNRGECDKTHTCPPCPAPEAAGGPSVFLFPPKPKDTLMISRTPEVTCVVVDVSHEDPEVKFNWYVDGVEVHNAKTKPREEQYNSTYRVVSVLTVLHQDWLNGKEYKCKVSNKALPAPIEKTISKAKGQPREPQVCTLPPSRDELTKNQVSLSCAVKGFYPSDIAVEWESNGQPENNYKTTPPVLDSDGSFFLVSKLTVDKSRWQQGNVFSCSVMHEALHNHYTQKSLSLSPGK

SEQ ID NO: 60 - protein, 443 aa, synthetic construct
QVQLVQSGAEVKKPGASVKVSCKASGYTFTGKWIEWVRQAPGQGLEWMGEILPGSGSTDYNERFKDRVTFTADTSTSTVYMELSSLRSEDTAVYYCVRSEDLWGQGTLVTVSSASTKGPSVFPLAPSSKSTSGGTAALGCLVKDYFPEPVTVSWNSGALTSGVHTFPAVLQSSGLYSLSSVVTVPSSSLGTQTYICNVNHKPSNTKVDKKVEPKSCDKTHTCPPCPAPEAAGGPSVFLFPPKPKDTLMISRTPEVTCVVVDVSHEDPEVKFNWYVDGVEVHNAKTKPREEQYNSTYRVVSVLTVLHQDWLNGKEYKCKVSNKALPAPIEKTISKAKGQPREPQVYTLPPCRDELTKNQVSLWCLVKGFYPSDIAVEWESNGQPENNYKTTPPVLDSDGSFFLYSKLTVDKSRWQQGNVFSCSVMHEALHNHYTQKSLSLSPGK

SEQ ID NO: 61 - protein, 443 aa, synthetic construct
QVQLVQSGAEVKKPGASVKVSCKASGYTFTGKWIEWVRQAPGQGLEWIGEILPGSGSTDYNERFKDRATFTADTSTSTAYMELSSLRSEDTAVYYCVRSEDLWGQGTLVTVSSASTKGPSVFPLAPSSKSTSGGTAALGCLVKDYFPEPVTVSWNSGALTSGVHTFPAVLQSSGLYSLSSVVTVPSSSLGTQTYICNVNHKPSNTKVDKKVEPKSCDKTHTCPPCPAPEAAGGPSVFLFPPKPKDTLMISRTPEVTCVVVDVSHEDPEVKFNWYVDGVEVHNAKTKPREEQYNSTYRVVSVLTVLHQDWLNGKEYKCKVSNKALPAPIEKTISKAKGQPREPQVYTLPPCRDELTKNQVSLWCLVKGFYPSDIAVEWESNGQPENNYKTTPPVLDSDGSFFLYSKLTVDKSRWQQGNVFSCSVMHEALHNHYTQKSLSLSPGK

SEQ ID NO: 62 - protein, 443 aa, synthetic construct
QVQLVQSGAEVKKPGASVKVSCKASGYTFTGKWIEWVRQAPGQGLEWMGEILPGSGSTDYNERFKDRATFTADTSTSTAYMELSSLRSEDTAVYYCVRSEDLWGQGTLVTVSSASTKGPSVFPLAPSSKSTSGGTAALGCLVKDYFPEPVTVSWNSGALTSGVHTFPAVLQSSGLYSLSSVVTVPSSSLGTQTYICNVNHKPSNTKVDKKVEPKSCDKTHTCPPCPAPEAAGGPSVFLFPPKPKDTLMISRTPEVTCVVVDVSHEDPEVKFNWYVDGVEVHNAKTKPREEQYNSTYRVVSVLTVLHQDWLNGKEYKCKVSNKALPAPIEKTISKAKGQPREPQVYTLPPCRDELTKNQVSLWCLVKGFYPSDIAVEWESNGQPENNYKTTPPVLDSDGSFFLYSKLTVDKSRWQQGNVFSCSVMHEALHNHYTQKSLSLSPGK

SEQ ID NO: 63 - protein, 10 aa, synthetic construct
GGGGSGGGGS

SEQ ID NO: 64 - protein, 20 aa, synthetic construct
GGGGSGGGGSGGGGSGGGGS

SEQ ID NO: 65 - protein, 15 aa, synthetic construct
GGGGSGGGGSGGGGS

SEQ ID NO: 66 - protein, 6 aa, synthetic construct
ASTKGP

SEQ ID NO: 67 - protein, 5 aa, synthetic construct
TVAAP

SEQ ID NO: 68 - protein, 17 aa, synthetic construct
EPKSDKTGGGGSGGGGS

SEQ ID NO: 69 - protein, 18 aa, synthetic construct
EPKSCGKTGGGGSGGGGS

SEQ ID NO: 70 - protein, 15 aa, synthetic construct
EPKSCGGGGSGGGGS

SEQ ID NO: 71 - protein, 24 aa, synthetic construct
GGGGSGGGGSEPKSDKTHTCPPCP

SEQ ID NO: 72 - protein, 15 aa, synthetic construct
GGGGSGGGGSCPPCP

SEQ ID NO: 73 - protein, 20 aa, synthetic construct
GGGGSGGGGSDKTHTCPPCP

SEQ ID NO: 74 - protein, 20 aa, synthetic construct
GKPGSGKPGSGKPGSGKPGS

SEQ ID NO: 75 - protein, 15 aa, synthetic construct
GGGGSGGGGTGGGGS

SEQ ID NO: 76 - protein, 22 aa, synthetic construct
GGGGSGGGGSESKYGPPCPPCP